European Patent Specification EP 4 003 394 B1, published April 16, 2025. Title: PEPTIDES FOR USE AS SENOTHERAPEUTIC AGENTS. Applicant: Fundación Profesor Novoa Santos, Universidade de Santiago de Compostela, Universidade da Coruña, Sevizo Galego de Saúde. The sequence listing filed with the application follows.

SEQUENCE LISTING (21 sequences)

SEQ ID NO: 1 - protein, 18 aa, Artificial sequence
  Artificial sequence
GKSDPYHATSGALSPAKD

SEQ ID NO: 2 - protein, 18 aa, Artificial sequence
  Artificial sequence
GKSDPYHATTGPLSPAKD

SEQ ID NO: 3 - protein, 11 aa, Artificial sequence
  Artificial sequence
FKGVKDRVKGK

SEQ ID NO: 4 - DNA, 22 bp, Artificial sequence
  Artificial sequence
ttgagtttggaaacatctggag

SEQ ID NO: 5 - DNA, 21 bp, Artificial sequence
  Artificial sequence
gcccaaagggaactgatagtc

SEQ ID NO: 6 - DNA, 20 bp, Artificial sequence
  Artificial sequence
gagcagaacgatagggcttg

SEQ ID NO: 7 - DNA, 20 bp, Artificial sequence
  Artificial sequence
catgtgccctctcctcctaa

SEQ ID NO: 8 - DNA, 20 bp, Artificial sequence
  Artificial sequence
gactctcagggtcgaaaacg

SEQ ID NO: 9 - DNA, 22 bp, Artificial sequence
  Artificial sequence
gccagggtatgtacaatgagga

SEQ ID NO: 10 - DNA, 20 bp, Artificial sequence
  Artificial sequence
ccctgggtctctttcactca

SEQ ID NO: 11 - DNA, 20 bp, Artificial sequence
  Artificial sequence
gctgacagcatcaaaggaca

SEQ ID NO: 12 - DNA, 18 bp, Artificial sequence
  Artificial sequence
catgtccgcgtcccacta

SEQ ID NO: 13 - DNA, 20 bp, Artificial sequence
  Artificial sequence
cacgccctgtttctttgaat

SEQ ID NO: 14 - DNA, 20 bp, Artificial sequence
  Artificial sequence
cagaacaactcggggaacat

SEQ ID NO: 15 - DNA, 20 bp, Artificial sequence
  Artificial sequence
gcacaattggaaccctgact

SEQ ID NO: 16 - DNA, 21 bp, Artificial sequence
  Artificial sequence
cgaatctccgaccaccactac

SEQ ID NO: 17 - DNA, 21 bp, Artificial sequence
  Artificial sequence
cgaatctccgaccaccactac

SEQ ID NO: 18 - DNA, 17 bp, Artificial sequence
  Artificial sequence
tgtagccgccccacaca

SEQ ID NO: 19 - DNA, 22 bp, Artificial sequence
  Artificial sequence
ggatgtaccgaatttgtttgta

SEQ ID NO: 20 - DNA, 21 bp, Artificial sequence
  Artificial sequence
cttcacgcatcagtttttcaa

SEQ ID NO: 21 - DNA, 26 bp, Artificial sequence
  Artificial sequence
tcaccgtaaatatgatttaagtccac